European Patent Specification EP 2 592 924 B1, published April 29, 2026. Title: SQUASH LEAF CURL VIRUS (SLCV) RESISTANCE IN CUCURBITS. Applicant: Superak, Ted. The sequence listing filed with the application follows.

SEQUENCE LISTING (26 sequences)

SEQ ID NO: 1 - DNA, 18 bp, Artificial Sequence
  E12/M49 F
gactgcgtaccaattcac

SEQ ID NO: 2 - DNA, 19 bp, Artificial Sequence
  E12/M49 R
gatgagtcctgagtaacag

SEQ ID NO: 3 - DNA, 18 bp, Artificial Sequence
  E12/M51 F
gactgcgtaccaattcac

SEQ ID NO: 4 - DNA, 19 bp, Artificial Sequence
  E12/M51 R
gatgagtcctgagtaacca

SEQ ID NO: 5 - DNA, 18 bp, Artificial Sequence
  E12/M58 F
gactgcgtaccaattcac

SEQ ID NO: 6 - DNA, 19 bp, Artificial Sequence
  E12/M58 R
gatgagtcctgagtaacgt

SEQ ID NO: 7 - DNA, 18 bp, Artificial Sequence
  E12/M62 F
gactgcgtaccaattcac

SEQ ID NO: 8 - DNA, 19 bp, Artificial Sequence
  E12/M62 R
gatgagtcctgagtaactt

SEQ ID NO: 9 - DNA, 18 bp, Artificial Sequence
  E14/M49 F
gactgcgtaccaattcat

SEQ ID NO: 10 - DNA, 19 bp, Artificial Sequence
  E14/M49 R
gatgagtcctgagtaacag

SEQ ID NO: 11 - DNA, 18 bp, Artificial Sequence
  E14/M58 F
gactgcgtaccaattcat

SEQ ID NO: 12 - DNA, 19 bp, Artificial Sequence
  E14/M58 R
gatgagtcctgagtaacgt

SEQ ID NO: 13 - DNA, 18 bp, Artificial Sequence
  E15/M60 F
gactgcgtaccaattcca

SEQ ID NO: 14 - DNA, 19 bp, Artificial Sequence
  E15/M60 R
gatgagtcctgagtaactc

SEQ ID NO: 15 - DNA, 18 bp, Artificial Sequence
  E15/M61 F
gactgcgtaccaattcca

SEQ ID NO: 16 - DNA, 19 bp, Artificial Sequence
  E15/M61 R
gatgagtcctgagtaactg

SEQ ID NO: 17 - DNA, 18 bp, Artificial Sequence
  E18/M54 F
gactgcgtaccaattcct

SEQ ID NO: 18 - DNA, 19 bp, Artificial Sequence
  E18/M54 R
gatgagtcctgagtaacct

SEQ ID NO: 19 - DNA, 18 bp, Artificial Sequence
  E18/M62 F
gactgcgtaccaattcct

SEQ ID NO: 20 - DNA, 19 bp, Artificial Sequence
  E18/M62 R
gatgagtcctgagtaactt

SEQ ID NO: 21 - DNA, 18 bp, Artificial Sequence
  E23/M48 F
gactgcgtaccaattcta

SEQ ID NO: 22 - DNA, 19 bp, Artificial Sequence
  E23/M48 R
gatgagtcctgagtaacac

SEQ ID NO: 23 - DNA, 18 bp, Artificial Sequence
  E23/M60 F
gactgcgtaccaattcta

SEQ ID NO: 24 - DNA, 19 bp, Artificial Sequence
  E23/M60 R
gatgagtcctgagtaactc

SEQ ID NO: 25 - DNA, 18 bp, Artificial Sequence
  E26/M48 F
gactgcgtaccaattctt

SEQ ID NO: 26 - DNA, 19 bp, Artificial Sequence
  E26/M48 R
gatgagtcctgagtaacac